European Patent Application EP 4 272 758 A1, published November 8, 2023. Title: Drug for alleviating neuropathic pain. Applicant: Asahi Kasei Pharma Corporation. The sequence listing filed with the application follows.

SEQUENCE LISTING (2 sequences)

SEQ ID NO: 1 - DNA, 1853 bp, Homo sapiens
  ref <308>: BC011913.2
aaaacgcagggagggaggctgtcaccatgccggcctgctgcagctgcagtgatgttttccagtatgagacgaacaaagtcactcggatccagagcatgaattatggcaccattaagtggttcttccacgtgatcatcttttcctacgtttgctttgctctggtgagtgacaagctgtaccagcggaaagagcctgtcatcagttctgtgcacaccaaggtgaaggggatagcagaggtgaaagaggagatcgtggagaatggagtgaagaagttggtgcacagtgtctttgacaccgcagactacaccttccctttgcaggggaactctttcttcgtgatgacaaactttctcaaaacagaaggccaagagcagcggttgtgtcccgagtatcccacccgcaggacgctctgttcctctgaccgaggttgtaaaaagggatggatggacccgcagagcaaaggaattcagaccggaaggtgtgtagtgcatgaagggaaccagaagacctgtgaagtctctgcctggtgccccatcgaggcagtggaagaggccccccggcctgctctcttgaacagtgccgaaaacttcactgtgctcatcaagaacaatatcgacttccccggccacaactacaccacgagaaacatcctgccaggtttaaacatcacttgtaccttccacaagactcagaatccacagtgtcccattttccgactaggagacatcttccgagaaacaggcgataatttttcagatgtggcaattcagggcggaataatgggcattgagatctactgggactgcaacctagaccgttggttccatcactgccatcccaaatacagtttccgtcgccttgacgacaagaccaccaacgtgtccttgtaccctggctacaacttcagatacgccaagtactacaaggaaaacaatgttgagaaacggactctgataaaagtcttcgggatccgttttgacatcctggtttttggcaccggaggaaaatttgacattatccagctggttgtgtacatcggctcaaccctctcctacttcggtctggccgctgtgttcatcgacttcctcatcgacacttactccagtaactgctgtcgctcccatatttatccctggtgcaagtgctgtcagccctgtgtggtcaacgaatactactacaggaagaagtgcgagtccattgtggagccaaagccgacattaaagtatgtgtcctttgtggatgaatcccacattaggatggtgaaccagcagctactagggagaagtctgcaagatgtcaagggccaagaagtcccaagacctgcgatggacttcacagatttgtccaggctgcccctggccctccatgacacacccccgattcctggacaaccagaggagatacagctgcttagaaaggaggcgactcctagatccagggatagccccgtctggtgccagtgtggaagctgcctcccatctcaactccctgagagccacaggtgcctggaggagctgtgctgccggaaaaagccgggggcctgcatcaccacctcagagctgttcaggaagctggtcctgtccagacacgtcctgcagttcctcctgctctaccaggagcccttgctggcgctggatgtggattccaccaacagccggctgcggcactgtgcctacaggtgctacgccacctggcgcttcggctcccaggacatggctgactttgccatcctgcccagctgctgccgctggaggatccggaaagagtttccgaagagtgaagggcagtacagtggcttcaagagtccttactgaagccaggcaccgtggctcacgtctgtaatcccacctttt

SEQ ID NO: 2 - protein, 595 aa, Homo sapiens
  ref <308>: AAH11913.1
MPACCSCSDVFQYETNKVTRIQSMNYGTIKWFFHVIIFSYVCFALVSDKLYQRKEPVISSVHTKVKGIAEVKEEIVENGVKKLVHSVFDTADYTFPLQGNSFFVMTNFLKTEGQEQRLCPEYPTRRTLCSSDRGCKKGWMDPQSKGIQTGRCVVHEGNQKTCEVSAWCPIEAVEEAPRPALLNSAENFTVLIKNNIDFPGHNYTTRNILPGLNITCTFHKTQNPQCPIFRLGDIFRETGDNFSDVAIQGGIMGIEIYWDCNLDRWFHHCHPKYSFRRLDDKTTNVSLYPGYNFRYAKYYKENNVEKRTLIKVFGIRFDILVFGTGGKFDIIQLVVYIGSTLSYFGLAAVFIDFLIDTYSSNCCRSHIYPWCKCCQPCVVNEYYYRKKCESIVEPKPTLKYVSFVDESHIRMVNQQLLGRSLQDVKGQEVPRPAMDFTDLSRLPLALHDTPPIPGQPEEIQLLRKEATPRSRDSPVWCQCGSCLPSQLPESHRCLEELCCRKKPGACITTSELFRKLVLSRHVLQFLLLYQEPLLALDVDSTNSRLRHCAYRCYATWRFGSQDMADFAILPSCCRWRIRKEFPKSEGQYSGFKSPY